European Patent Specification EP 3 784 803 B1, published February 11, 2026. Title: HLA-J and medical/diagnostic uses thereof. Applicant: Intellexon GmbH. The sequence listing filed with the application follows.

SEQUENCE LISTING (108 sequences)

SEQ ID NO: 1 - protein, 219 aa, Homo sapiens
  HLA-J protein
MAPRTLLLLLSGTLALAETWAGSHSMRYFSTAVSWPGRGEPSFIAVGYVDDTQFVRVDSDAVSLRMKTRARWVEQEGPEYWDLQTLGAKAQAQTDRVNLRTLLRYYNQSEADPPQDTRDPPPSLNMRHNEVLGSGLLPCGDHIDLAAGWGGPDPGHGARGDQAHRGWNLPEVGGCGSAFWRGTEIHMPCAAQGAAQAPHPEMGHTFLETSQGSKTRRFL

SEQ ID NO: 2 - DNA, 660 bp, Homo sapiens
  HLA-J ORF3
atggcgccccgaaccctcctcctgctgctctcggggaccctggccctggccgagacctgggcgggctcccactccatgaggtatttcagcaccgccgtttcctggccgggccgcggggagcccagcttcattgccgtgggctacgtggacgacacgcagttcgtgcgggtcgacagtgacgccgtgagtctgaggatgaagacgcgggcgcggtgggtggagcaggaggggccggagtattgggacctacagacactgggcgccaaggcccaggcacagactgaccgagtgaacctgcggaccctgctccgctactacaaccagagcgaggcggaccccccccaagacacacgtgacccacccccctctctgaacatgaggcataacgaggtcctgggttctgggcttctaccctgcggagatcacattgacctggcagcgggatggggaggaccagacccaggacatggagctcgtggagaccaggcccacaggggatggaaccttccagaagtgggcggttgtggtagtgccttctggagaggaacagagatacacatgccatgtgcagcacaaggggctgcccaagcccctcatcctgagatgggtcacacatttctggaaacttctcaaggttccaagactaggaggttcctctag

SEQ ID NO: 3 - DNA, 16 bp, Homo sapiens
  HLA-J unique 16 nucleotides insertion
tcacacatttctggaa

SEQ ID NO: 4 - DNA, 49 bp, Homo sapiens
  HLA-J unique 3‘-end
tcacacatttctggaaacttctcaaggttccaagactaggaggttcctc

SEQ ID NO: 5 - protein, 16 aa, Homo sapiens
  HLA-J unique C-terminal end
HTFLETSQGSKTRRFL

SEQ ID NO: 6 - DNA, 270 bp, Homo sapiens
  HLA-J alpha chain domain alpha 1 nucleotide sequence
ggctcccactccatgaggtatttcagcaccgccgtttcctggccgggccgcggggagcccagcttcattgccgtgggctacgtggacgacacgcagttcgtgcgggtcgacagtgacgccgtgagtctgaggatgaagacgcgggcgcggtgggtggagcaggaggggccggagtattgggacctacagacactgggcgccaaggcccaggcacagactgaccgagtgaacctgcggaccctgctccgctactacaaccagagcgaggcg

SEQ ID NO: 7 - DNA, 276 bp, Homo sapiens
  HLA-J alpha chain domain alpha 3 nucleotide sequence
gaccccccccaagacacacgtgacccacccccctctctgaacatgaggcataacgaggtcctgggttctgggcttctaccctgcggagatcacattgacctggcagcgggatggggaggaccagacccaggacatggagctcgtggagaccaggcccacaggggatggaaccttccagaagtgggcggttgtggtagtgccttctggagaggaacagagatacacatgccatgtgcagcacaaggggctgcccaagcccctcatcctgagatgggt

SEQ ID NO: 8 - protein, 90 aa, Homo sapiens
  HLA-J alpha chain domain alpha 1 amino acid sequence
GSHSMRYFSTAVSWPGRGEPSFIAVGYVDDTQFVRVDSDAVSLRMKTRARWVEQEGPEYWDLQTLGAKAQAQTDRVNLRTLLRYYNQSEA

SEQ ID NO: 9 - protein, 92 aa, Homo sapiens
  HLA-J alpha chain domain alpha 3 amino acid sequence
DPPQDTRDPPPSLNMRHNEVLGSGLLPCGDHIDLAAGWGGPDPGHGARGDQAHRGWNLPEVGGCGSAFWRGTEIHMPCAAQGAAQAPHPEMG

SEQ ID NO: 10 - DNA, 25 bp, Homo sapiens
  Consensus start site
atgggggtcatggcgccccgaaccc

SEQ ID NO: 11 - DNA, 24 bp, Homo sapiens
  Frame shift start site
atggggtcatggcgccccgaaccc

SEQ ID NO: 12 - DNA, 24 bp, Artificial Sequence
  HLA-J Forward Primer
cctctgtctctacacctccattcc

SEQ ID NO: 13 - DNA, 19 bp, Artificial Sequence
  HLA-J Forward Primer
ccctctctggcaccaagct

SEQ ID NO: 14 - DNA, 21 bp, Artificial Sequence
  HLA-J Forward Primer
gaccctgctccgctactacaa

SEQ ID NO: 15 - DNA, 17 bp, Artificial Sequence
  HLA-J Forward Primer
accccccccaagacaca

SEQ ID NO: 16 - DNA, 20 bp, Artificial Sequence
  HLA-J Forward Primer
gaccagacccaggacatgga

SEQ ID NO: 17 - DNA, 17 bp, Artificial Sequence
  HLA-J Forward Primer
tgcccaagcccctcatc

SEQ ID NO: 18 - DNA, 17 bp, Artificial Sequence
  HLA-J Forward Primer
tgcccaagcccctcatc

SEQ ID NO: 19 - DNA, 24 bp, Artificial Sequence
  HLA-J Forward Primer
ggaaacttctcaaggttccaagac

SEQ ID NO: 20 - DNA, 21 bp, Artificial Sequence
  HLA-J Forward Primer
ggagctactctcaggctgcaa

SEQ ID NO: 21 - DNA, 20 bp, Artificial Sequence
  HLA-J Forward Primer
tgccttgtgtgggactgaga

SEQ ID NO: 22 - DNA, 20 bp, Artificial Sequence
  HLA-J Forward Primer
cttccccgatcacctttcct

SEQ ID NO: 23 - DNA, 17 bp, Artificial Sequence
  HLA-J Forward Primer
gctctcggggaccctgg

SEQ ID NO: 24 - DNA, 17 bp, Artificial Sequence
  HLA-J Forward Primer
ccaatcagcgtcgcgcg

SEQ ID NO: 25 - DNA, 20 bp, Artificial Sequence
  CALM2 Forward Primer
gagcgagctgagtggttgtg

SEQ ID NO: 26 - DNA, 25 bp, Artificial Sequence
  HLA-J Probe
agctccctctctggcaccaagctcc

SEQ ID NO: 27 - DNA, 24 bp, Artificial Sequence
  HLA-J Probe
agcctgcgacgggtccttcttcct

SEQ ID NO: 28 - DNA, 20 bp, Artificial Sequence
  HLA-J Probe
cagagcgaggcggacccccc

SEQ ID NO: 29 - DNA, 25 bp, Artificial Sequence
  HLA-J Probe
tgacccacccccctctctgaacatg

SEQ ID NO: 30 - DNA, 23 bp, Artificial Sequence
  HLA-J Probe
ctcgtggagaccaggcccacagg

SEQ ID NO: 31 - DNA, 32 bp, Artificial Sequence
  HLA-J Probe
tgagatgggtcacacatttctggaaacttctc

SEQ ID NO: 32 - DNA, 32 bp, Artificial Sequence; identical to SEQ ID NO: 31
  HLA-J Probe

SEQ ID NO: 33 - DNA, 28 bp, Artificial Sequence
  HLA-J Probe
aggttcctctaggacctcatggccctgc

SEQ ID NO: 34 - DNA, 21 bp, Artificial Sequence
  HLA-J Probe
cagccaaagtgcccagggctc

SEQ ID NO: 35 - DNA, 30 bp, Artificial Sequence
  HLA-J Probe
caagatttgttcatgccttccctttgtgac

SEQ ID NO: 36 - DNA, 28 bp, Artificial Sequence
  HLA-J Probe
cagagaagtggtgctgggatgtctccat

SEQ ID NO: 37 - DNA, 26 bp, Artificial Sequence
  HLA-J Probe
atgaggtatttcagcaccgccgttcc

SEQ ID NO: 38 - DNA, 23 bp, Artificial Sequence
  HLA-J Probe
acgcacccaccgggactcggagt

SEQ ID NO: 39 - DNA, 22 bp, Artificial Sequence
  CALM2 Probe
tcgcgtctcggaaaccggtagc

SEQ ID NO: 40 - DNA, 22 bp, Artificial Sequence
  HLA-J Reverse Primer
ttcccctggactcttcaaaaag

SEQ ID NO: 41 - DNA, 18 bp, Artificial Sequence
  HLA-J Reverse Primer
ggtccgcgtcgtgagtgt

SEQ ID NO: 42 - DNA, 22 bp, Artificial Sequence
  HLA-J Reverse Primer
agaacccaggacctcgttatgc

SEQ ID NO: 43 - DNA, 21 bp, Artificial Sequence
  HLA-J Reverse Primer
gaacccaggacctcgttatgc

SEQ ID NO: 44 - DNA, 20 bp, Artificial Sequence
  HLA-J Reverse Primer
taccacaaccgcccacttct

SEQ ID NO: 45 - DNA, 20 bp, Artificial Sequence
  HLA-J Reverse Primer
cagggccatgaggtcctaga

SEQ ID NO: 46 - DNA, 26 bp, Artificial Sequence
  HLA-J Reverse Primer
ctagaggaacctcctagtcttggaac

SEQ ID NO: 47 - DNA, 21 bp, Artificial Sequence
  HLA-J Reverse Primer
ctgtgagaggccaggaaggta

SEQ ID NO: 48 - DNA, 24 bp, Artificial Sequence
  HLA-J Reverse Primer
ctttacaagccgtgagagacacat

SEQ ID NO: 49 - DNA, 25 bp, Artificial Sequence
  HLA-J Reverse Primer
cagaaagagaagtcagggttcttga

SEQ ID NO: 50 - DNA, 23 bp, Artificial Sequence
  HLA-J Reverse Primer
tacagctcagtgcaccatgaagt

SEQ ID NO: 51 - DNA, 18 bp, Artificial Sequence
  HLA-J Reverse Primer
cccacggcaatgaagctg

SEQ ID NO: 52 - DNA, 17 bp, Artificial Sequence
  HLA-J Reverse Primer
accccatcgtcggcgtc

SEQ ID NO: 53 - DNA, 21 bp, Artificial Sequence
  CALM2 Reverse Primer
agtcagttggtcagccatgct

SEQ ID NO: 54 - protein, 5 aa, Artificial Sequence
  GS-Linker
GGGGS

SEQ ID NO: 55 - protein, 4 aa, Artificial Sequence
  Variable loop
CGPC

SEQ ID NO: 56 - DNA, 18 bp, Artificial Sequence
  RPL37A Probe
tggctggcggtgcctgga

SEQ ID NO: 57 - DNA, 28 bp, Artificial Sequence
  GAPDH Probe
aaggtgaaggtcggagtcaacggatttg

SEQ ID NO: 58 - DNA, 19 bp, Artificial Sequence
  ESR1 Probe
atgcccttttgccgatgca

SEQ ID NO: 59 - DNA, 19 bp, Artificial Sequence
  ESR1 Probe
ctggagatgctggacgccc

SEQ ID NO: 60 - DNA, 26 bp, Artificial Sequence
  MLPH Probe
ccaaatgcagacccttcaagtgaggc

SEQ ID NO: 61 - DNA, 28 bp, Artificial Sequence
  MLPH Probe
cgggcgtcttctgagagtcagatctttg

SEQ ID NO: 62 - DNA, 22 bp, Artificial Sequence
  ERBB2 Probe
aggccaagtccgcagaagccct

SEQ ID NO: 63 - DNA, 31 bp, Artificial Sequence
  ERBB2 Probe
tgatcatggtcaaatgttggatgattgactc

SEQ ID NO: 64 - DNA, 32 bp, Artificial Sequence
  MMP1 Probe
agagagtacaacttacatcgtgttgcggctca

SEQ ID NO: 65 - DNA, 30 bp, Artificial Sequence
  MMP1 Probe
acagagatgaagtccggtttttcaaaggga

SEQ ID NO: 66 - DNA, 28 bp, Artificial Sequence
  MMP7 Probe
cagtctagggattaacttcctgtatgct

SEQ ID NO: 67 - DNA, 31 bp, Artificial Sequence
  MMP7 Probe
agtgggaacaggctcaggactatctcaagag

SEQ ID NO: 68 - DNA, 24 bp, Artificial Sequence
  KRT5 Probe
tggagggcgaggaatgcagactca

SEQ ID NO: 69 - DNA, 21 bp, Artificial Sequence
  RPL37A Forward Primer
tgtggttcctgcatgaagaca

SEQ ID NO: 70 - DNA, 17 bp, Artificial Sequence
  GAPDH Forward Primer
gccagccgagccacatc

SEQ ID NO: 71 - DNA, 24 bp, Artificial Sequence
  ESR1 Forward Primer
gccaaattgtgtttgatggattaa

SEQ ID NO: 72 - DNA, 19 bp, Artificial Sequence
  ESR1 Forward Primer
cgtggtgcccctctatgac

SEQ ID NO: 73 - DNA, 20 bp, Artificial Sequence
  MLPH Forward Primer
tcgagtggctgggaaacttg

SEQ ID NO: 74 - DNA, 21 bp, Artificial Sequence
  MLPH Forward Primer
cgatgtggacacctctgatga

SEQ ID NO: 75 - DNA, 20 bp, Artificial Sequence
  ERBB2 Forward Primer
tctggacgtgccagtgtgaa

SEQ ID NO: 76 - DNA, 23 bp, Artificial Sequence
  ERBB2 Forward Primer
ccatctgcaccattgatgtctac

SEQ ID NO: 77 - DNA, 24 bp, Artificial Sequence
  MMP1 Forward Primer
agatgaaaggtggaccaacaattt

SEQ ID NO: 78 - DNA, 22 bp, Artificial Sequence
  MMP1 Forward Primer
ttgaagctgcttacgaatttgc

SEQ ID NO: 79 - DNA, 19 bp, Artificial Sequence
  MMP7 Forward Primer
gaacgctggacggatggta

SEQ ID NO: 80 - DNA, 20 bp, Artificial Sequence
  MMP7 Forward Primer
cgggaggcatgagtgagcta

SEQ ID NO: 81 - DNA, 18 bp, Artificial Sequence
  KRT5 Forward Primer
cgccacttaccgcaagct

SEQ ID NO: 82 - DNA, 24 bp, Artificial Sequence
  RPL37A Reverse Primer
gtgacagcggaagtggtattgtac

SEQ ID NO: 83 - DNA, 15 bp, Artificial Sequence
  GAPDH Reverse Primer
ccaggcgcccaatag

SEQ ID NO: 84 - DNA, 27 bp, Artificial Sequence
  ESR1 Reverse Primer
gacaaaaccgagtcacatcagtaatag

SEQ ID NO: 85 - DNA, 19 bp, Artificial Sequence
  ESR1 Reverse Primer
ggctagtgggcgcatgtag

SEQ ID NO: 86 - DNA, 20 bp, Artificial Sequence
  MLPH Reverse Primer
agatagggcacagccattgc

SEQ ID NO: 87 - DNA, 23 bp, Artificial Sequence
  MLPH Reverse Primer
aggcattccacagctgaaatatg

SEQ ID NO: 88 - DNA, 20 bp, Artificial Sequence
  ERBB2 Reverse Primer
cctgctccctgaggacacat

SEQ ID NO: 89 - DNA, 19 bp, Artificial Sequence
  ERBB2 Reverse Primer
cggaatcttggccgacatt

SEQ ID NO: 90 - DNA, 20 bp, Artificial Sequence
  MMP1 Reverse Primer
ccaagagaatggccgagttc

SEQ ID NO: 91 - DNA, 23 bp, Artificial Sequence
  MMP1 Reverse Primer
gtccctgaacagcccagtactta

SEQ ID NO: 92 - DNA, 22 bp, Artificial Sequence
  MMP7 Reverse Primer
gaatggccaagttcatgagttg

SEQ ID NO: 93 - DNA, 26 bp, Artificial Sequence
  MMP7 Reverse Primer
ggcattttttgtttctgagtcataga

SEQ ID NO: 94 - DNA, 25 bp, Artificial Sequence
  KRT5 Reverse Primer
acagagatgttgactggtccaactc

SEQ ID NO: 95 - DNA, 177 bp, Homo sapiens
  NM_001098479.1
cacgcaccccgcgggactcatatttttcccagacgcggaggttggggtcatggcgccccgaagcctcctcctgctgctctcaggggccctggccctgaccgatacttgggcgggctcccactccttgaggtatttcagcaccgctgtgtgcggcccggccgcggggagccccgctac

SEQ ID NO: 96 - DNA, 178 bp, Homo sapiens
  NM_018950.2
cacgcaccccgcgggactcatatttttcccagacgcggaggttggggtcatggcgccccgaagcctcctcctgctgctctcaggggccctggccctgaccgatacttgggcgggctcccactccttgaggtatttcagcaccgctgtgtcgcggcccggccgcggggagccccgctac

SEQ ID NO: 97 - DNA, 178 bp, Homo sapiens; identical to SEQ ID NO: 96
  NM_001098478.1

SEQ ID NO: 98 - DNA, 179 bp, Homo sapiens
  NR_024240.1
ccacgcacccaccgggactcggagtctccccagacgccgacgatggggtcatggcgccccgaaccctcctcctgctgctctcggggaccctggccctggccgagacctgggcgggctcccactccatgaggtatttcagcaccgccgtttcctggccgggccgcggggagcccagcttc

SEQ ID NO: 99 - DNA, 178 bp, Homo sapiens
  NM_002127.5
tcgctcacccacccggactcattctccccagacgccaaggatggtggtcatggcgccccgaaccctcttcctgctgctctcgggggccctgaccctgaccgagacctgggcgggctcccactccatgaggtatttcagcgccgccgtgtcccggcccggccgcggggagccccgcttc

SEQ ID NO: 100 - DNA, 180 bp, Homo sapiens
  NM_002116.7
gcacgcacccaccgggactcagattctccccagacgccgaggatggccgtcatggcgccccgaaccctcctcctgctactctcgggggccctggccctgacccagacctgggcgggctcccactccatgaggtatttcttcacatccgtgtcccggcccggccgcggggagccccgcttc

SEQ ID NO: 101 - DNA, 180 bp, Homo sapiens; identical to SEQ ID NO: 100
  NM_001242758.1

SEQ ID NO: 102 - DNA, 159 bp, Homo sapiens
  NM_001098479.1
cacgaggggctgccccagcccctcatcctgagatgggagcagtctccccagcccaccatccccatcgtgggcatgttgctggccttgttgtccttggagctgtggtcactggagctgtggtcgctgctgtgatgtggaggaagaagagctcagatagaa

SEQ ID NO: 103 - DNA, 160 bp, Homo sapiens
  NM_018950.2
cacgaggggctgccccagcccctcatcctgagatgggagcagtctccccagcccaccatccccatcgtgggcatcgttgctggccttgttgtccttggagctgtggtcactggagctgtggtcgctgctgtgatgtggaggaagaagagctcagatagaa

SEQ ID NO: 104 - DNA, 123 bp, Homo sapiens
  NM_001098478.1
agcagtctccccagcccaccatccccatcgtgggcatcgttgctggccttgttgtccttggagctgtggtcactggagctgtggtcgctgctgtgatgtggaggaagaagagctcagatagaa

SEQ ID NO: 105 - DNA, 150 bp, Homo sapiens
  NR_024240.1
cacaaggggctgcccaagcccctcatcctgagatgggtcacacatttctggaaacttctcaaggttccaagactaggaggttcctctaggacctcatggccctgctaccttcctggcctctcacaggacgttttcttcccgcagatagaa

SEQ ID NO: 106 - DNA, 160 bp, Homo sapiens
  NM_002127.5
catgaggggctgccggagcccctcatgctgagatggaagcagtcttccctgcccaccatccccatcatgggtatcgttgctggcctggttgtccttgcagctgtagtcactggagctgcggtcgctgctgtgctgtggagaaagaagagctcagattgaa

SEQ ID NO: 107 - DNA, 160 bp, Homo sapiens
  NM_002116.7
catgagggtctgcccaagcccctcaccctgagatgggagctgtcttcccagcccaccatccccatcgtgggcatcattgctggcctggttctccttggagctgtgatcactggagctgtggtcgctgccgtgatgtggaggaggaagagctcagatagaa

SEQ ID NO: 108 - DNA, 160 bp, Homo sapiens; identical to SEQ ID NO: 107
  NM_001242758.1